European Patent Specification EP 4 447 988 B1, published May 27, 2026. Title: Compositions for treating autoimmune arthritis. Applicant: DEVINTEC SAGL. The sequence listing filed with the application follows.

SEQUENCE LISTING (6 sequences)

SEQ ID NO: 1 - DNA, 20 bp, synthetic construct
  source 1..20: mol_type = other DNA
tgattccgcatggtttcatt

SEQ ID NO: 2 - DNA, 20 bp, synthetic construct
  source 1..20: mol_type = other DNA
cgacccatagagccttcatc

SEQ ID NO: 3 - DNA, 16 bp, synthetic construct
  source 1..16: mol_type = other DNA
cccgacgggaggggat

SEQ ID NO: 4 - DNA, 22 bp, synthetic construct
  source 1..22: mol_type = other DNA
cttctgcaggtacagtcttgac

SEQ ID NO: 5 - DNA, 17 bp, synthetic construct
  source 1..17: mol_type = other DNA
cagcagccgcggtaata

SEQ ID NO: 6 - DNA, 19 bp
ggcatccatcgtttaccgt